European Patent Application EP 4 628 511 A1, published October 8, 2025. Title: 重组血红蛋白. Applicant: 康码（上海）生物科技有限公司. The sequence listing filed with the application follows.

SEQUENCE LISTING (16 sequences)

SEQ ID NO: 1 - protein, 26 aa, synthetic construct
GGGGSRADARADARADARADAGGGGS

SEQ ID NO: 2 - protein, 22 aa, synthetic construct
GGGGSKLDLKLDLKLDLGGGGS

SEQ ID NO: 3 - protein, 22 aa, synthetic construct
GGGGSLKLKLKLKLKLKGGGGS

SEQ ID NO: 4 - protein, 22 aa, synthetic construct
GGGGSLDLDLDLDLDLDGGGGS

SEQ ID NO: 5 - protein, 10 aa, synthetic construct
GGGGSGGGGS

SEQ ID NO: 6 - protein, 20 aa, synthetic construct
GGGGSGGGGSGGGGSGGGGS

SEQ ID NO: 7 - protein, 141 aa, synthetic construct
VLSPADKTNVKAAWAKVGAHAGEYGAEAFERMFLSFPTTKTYFPHFDLSHGSAQVKGQGKKVADALTNAVAHVDDMPNALSALSDLHAHKLRVDPWNFKLLSHCLLVTLAAHLPAEFTPAVHASLDKFLASVSTVLTSKYR

SEQ ID NO: 8 - protein, 146 aa, synthetic construct
VHLTPEEKSAVTALWAKVNVDEVGGEALGRLLVVYPWTQRFFEHFGDLSTPDAVMGNPKVKAHGKKVLGAFSDGLAHLDNLDGTFATLSELHCDKLHVDPENFRLLGNVLVCVLAIHFGKEFTPPVQAAYQKVVAGVANALAHKYH

SEQ ID NO: 9 - protein, 238 aa, synthetic construct
VSKGEELFTGVVPILVELDGDVNGHKFSVRGEGEGDATNGKLTLKFICTTGKLPVPWPTLVTTLTYGVQCFSRYPDHMKQHDFFKSAMPEGYVQERTISFKDDGTYKTRAEVKFEGDTLVNRIELKGIDFKEDGNILGHKLEYNFNSHNVYITADKQKNGIKANFKIRHNVEDGSVQLADHYQQNTPIGDGPVLLPDNHYLSTQSKLSKDPNEKRDHMVLLEFVTAAGITLGMDELYK

SEQ ID NO: 10 - protein, 34 aa, synthetic construct
SGGGSGGGSEGGGSEGGGSEGGGSEGGGSGGGSG

SEQ ID NO: 11 - protein, 60 aa, synthetic construct
GGSSGSGSGSTGTSSSGTGTSAGTTGTSASTSGSGSGGGGGSGGGGSAGGTATAGASSGS

SEQ ID NO: 12 - protein, 81 aa, synthetic construct
GGSSGSGSGSTGTSSSGTGTSAGTTGTSASTSGSGSGGGGGSGGGGSAGGTATAGAGSTGGAGSTGGAGSTGGAGTGSGAG

SEQ ID NO: 13 - protein, 141 aa, synthetic construct
VLSAADKGNVKAAWGKVGGHAAEYGAEALERMFLSFPTTKTYFPHFDLSHGSAQVKGHGAKVAAALTKAVEHLDDLPGALSELSDLHAHKLRVDPVNFKLLSHSLLVTLASHLPSDFTPAVHASLDKFLANVSTVLTSKYR

SEQ ID NO: 14 - protein, 141 aa, synthetic construct
VLSAADKANVKAAWGKVGGQAGAHGAEALERMFLGFPTTKTYFPHFNLSHGSDQVKAHGQKVADALTKAVGHLDDLPGALSALSDLHAHKLRVDPVNFKLLSHCLLVTLAAHHPDDFNPSVHASLDKFLANVSTVLTSKYR

SEQ ID NO: 15 - protein, 144 aa, synthetic construct
LTAEEKAAVTAFWGKVKVDEVGGEALGRLLVVYPWTQRFFESFGDLSTADAVMNNPKVKAHGKKVLDSFSNGMKHLDDLKGTFAALSELHCDKLHVDPENFKLLGNVLVVVLARNFGKEFTPVLQADFQKVVAGVANALAHRYH

SEQ ID NO: 16 - protein, 146 aa, synthetic construct
VHLSAEEKEAVLGLWGKVNVDEVGGEALGRLLVVYPWTQRFFESFGDLSNADAVMGNPKVKAHGKKVLQSFSDGLKHLDNLKGTFAKLSELHCDQLHVDPENFRLLGNVIVVVLARRLGHDFNPNVQAAFQKVVAGVANALAHKYH